European Patent Application EP 4 223 771 A1, published August 9, 2023. Title: SCREENING AND ANTITUMOR USE OF KRAS MUTATION SPECIFIC T CELL RECEPTOR. Applicant: Institute of Microbiology, Chinese Academy of Sciences. Application EP21874505.7. The sequence listing filed with the application follows.

SEQUENCE LISTING (48 sequences)

SEQ ID NO: 1 - DNA, 333 bp, Artificial Sequence
  Artificially synthesized sequence
gccaacagaaggtgcagcagagcccagaatccctcattgttccagagggaggcatggcctctctcaactgcacttccagtgatcgtaatgttgactacttctggtggtacagacagcactctgggaaaagccccaagatgctgatgtctatcttctccaatggtgaaaaggaagaaggcagattcacagttcacctcaataaagccagcctgcatacttccctgcacatcagagactcccagcccagtgactctgctctctacctctgtgcagcaagggacagcaactatcagttgatctggggctctgggaccaagctaattataaagccag

SEQ ID NO: 2 - protein, 111 aa, Artificial Sequence
  Artificially synthesized sequence
QQKVQQSPESLIVPEGGMASLNCTSSDRNVDYFWWYRQHSGKSPKMLMSIFSNGEKEEGRFTVHLNKASLHTSLHIRDSQPSDSALYLCAARDSNYQLIWGSGTKLIIKPD

SEQ ID NO: 3 - protein, 6 aa, Artificial Sequence
  Artificially synthesized sequence
DRNVDY

SEQ ID NO: 4 - protein, 6 aa, Artificial Sequence
  Artificially synthesized sequence
IFSNGE

SEQ ID NO: 5 - protein, 10 aa, Artificial Sequence
  Artificially synthesized sequence
AARDSNYQLI

SEQ ID NO: 6 - DNA, 336 bp, Artificial Sequence
  Artificially synthesized sequence
aggctgcagtcacccaaagcccaagaaacaaggtggcagtaacaggaggaaaggtgacattgagctgtaatcagactaataaccacaacaacatgtactggtatcggcaggacacggggcatgggctgaggctgatccattattcatatggtgctggcagcactgagaaaggagatatccctgatggatacaaggcctccagaccaagccaagagaacttctccctcattctggagttggctaccccctctcagacatcagtgtacttctgtgccagcggtgatacagggggctatgaacagtacttcggtcccggcaccaggctcacggttttag

SEQ ID NO: 7 - protein, 112 aa, Artificial Sequence
  Artificially synthesized sequence
EAAVTQSPRNKVAVTGGKVTLSCNQTNNHNNMYWYRQDTGHGLRLIHYSYGAGSTEKGDIPDGYKASRPSQENFSLILELATPSQTSVYFCASGDTGGYEQYFGPGTRLTVL

SEQ ID NO: 8 - protein, 5 aa, Artificial Sequence
  Artificially synthesized sequence
NNHNN

SEQ ID NO: 9 - protein, 6 aa, Artificial Sequence
  Artificially synthesized sequence
SYGAGS

SEQ ID NO: 10 - protein, 11 aa, Artificial Sequence
  Artificially synthesized sequence
ASGDTGGYEQY

SEQ ID NO: 11 - DNA, 328 bp, Artificial Sequence
  Artificially synthesized sequence
caactagcagaagagaattcgtgggccctgagcgtccacgagggtgaaagtgtcacggtgaattgtagttacaagacatccataactgccctacagtggtacagacagaagtcaggcaaaggccctgcccagctaatcttaatacgttcaaatgagagagagaagcgcaatggaagactcagagccacccttgacacctccagccagagcagctccttgtccatcactgctactcggtgtgaagacaccgctgtgtacttctgtgccgcatcttctggcagctggcaactcatctttggatctggaacccaactgacagttatgcctg

SEQ ID NO: 12 - protein, 109 aa, Artificial Sequence
  Artificially synthesized sequence
QLAEENSWALSVHEGESVTVNCSYKTSITALQWYRQKSGKGPAQLILIRSNEREKRNGRLRATLDTSSQSSSLSITATRCEDTAVYFCAASSGSWQLIFGSGTQLTVMP

SEQ ID NO: 13 - protein, 5 aa, Artificial Sequence
  Artificially synthesized sequence
TSITA

SEQ ID NO: 14 - protein, 7 aa, Artificial Sequence
  Artificially synthesized sequence
IRSNERE

SEQ ID NO: 15 - protein, 10 aa, Artificial Sequence
  Artificially synthesized sequence
AASSGSWQLI

SEQ ID NO: 16 - DNA, 346 bp, Artificial Sequence
  Artificially synthesized sequence
aatgctggtgtcatccaaacacctaggcacaaggtgacagggaagggacaagaagcaactctgtggtgtgagccaatttcaggacatagtgctgttttctggtacagacagaccattgtgcagggcctggagttcctgacttactttcgaaatcaagctcctatagatgattcagggatgcccaaggaacgattctcagctcagatgcccaatcagtcgcactcaactctgaagatccagagcacgcaaccccaggactcagcggtgtatctttgtgcaagcagcttagaagggacagtggaagaaacgctgtattttggctcaggaaccagactgactgttctcg

SEQ ID NO: 17 - protein, 115 aa, Artificial Sequence
  Artificially synthesized sequence
NAGVIQTPRHKVTGKGQEATLWCEPISGHSAVFWYRQTIVQGLEFLTYFRNQAPIDDSGMPKERFSAQMPNQSHSTLKIQSTQPQDSAVYLCASSLEGTVEETLYFGSGTRLTVL

SEQ ID NO: 18 - protein, 5 aa, Artificial Sequence
  Artificially synthesized sequence
SGHSA

SEQ ID NO: 19 - protein, 6 aa, Artificial Sequence
  Artificially synthesized sequence
FRNQAP

SEQ ID NO: 20 - protein, 13 aa, Artificial Sequence
  Artificially synthesized sequence
ASSLEGTVEETLY

SEQ ID NO: 21 - DNA, 813 bp, Artificial Sequence
  Artificially synthesized sequence
atgaaatcctttagtatttccctagtggtcctgtggcttcagctaaactgggtgaacagccaacagaaggtgcagcagagcccagaatccctcattgttccagagggaggcatggcctctctcaactgcacttccagtgatcgtaatgttgactacttctggtggtacagacagcactctgggaaaagccccaagatgctgatgtctatcttctccaatggtgaaaaggaagaaggcagattcacagttcacctcaataaagccagcctgcatacttccctgcacatcagagactcccagcccagtgactctgctctctacctctgtgcagcaagggacagcaactatcagttgatctggggctctgggaccaagctaattataaagccagatatccagaaccctgaccctgccgtgtaccagctgagagactctaaatccagtgacaagtctgtctgcctattcaccgattttgattctcaaacaaatgtgtcacaaagtaaggattctgatgtgtatatcacagacaaatgcgtgctagacatgaggtctatggacttcaagagcaacagtgctgtggcctggagcaacaaatctgactttgcatgtgcaaacgccttcaacaacagcattattccagaagacaccttcttccccagcccagaaagttcctgtgatgtcaagctggtcgagaaaagctttgaaacagatacgaacctaaactttcaaaacctgtcagtgattgggttccgaatcctcctcctgaaagtggccgggtttaatctgctcatgacgctgcggctgtggtccagc

SEQ ID NO: 22 - protein, 271 aa, Artificial Sequence
  Artificially synthesized sequence
MKSFSISLVVLWLQLNWVNSQQKVQQSPESLIVPEGGMASLNCTSSDRNVDYFWWYRQHSGKSPKMLMSIFSNGEKEEGRFTVHLNKASLHTSLHIRDSQPSDSALYLCAARDSNYQLIWGSGTKLIIKPDIQNPDPAVYQLRDSKSSDKSVCLFTDFDSQTNVSQSKDSDVYITDKCVLDMRSMDFKSNSAVAWSNKSDFACANAFNNSIIPEDTFFPSPESSCDVKLVEKSFETDTNLNFQNLSVIGFRILLLKVAGFNLLMTLRLWSS

SEQ ID NO: 23 - DNA, 927 bp, Artificial Sequence
  Artificially synthesized sequence
atgggctccaggctcttcttcgtgctctccagtctcctgtgttcaaaacacatggaggctgcagtcacccaaagcccaagaaacaaggtggcagtaacaggaggaaaggtgacattgagctgtaatcagactaataaccacaacaacatgtactggtatcggcaggacacggggcatgggctgaggctgatccattattcatatggtgctggcagcactgagaaaggagatatccctgatggatacaaggcctccagaccaagccaagagaacttctccctcattctggagttggctaccccctctcagacatcagtgtacttctgtgccagcggtgatacagggggctatgaacagtacttcggtcccggcaccaggctcacggttttagaggacctgaaaaacgtgttcccacccgaggtcgctgtgtttgagccatcagaagcagagatctcccacacccaaaaggccacactggtgtgcctggccacaggcttctaccccgaccacgtggagctgagctggtgggtgaatgggaaggaggtgcacagtggggtctgcacagacccgcagcccctcaaggagcagcccgccctcaatgactccagatactgcctgagcagccgcctgagggtctcggccaccttctggcagaacccccgcaaccacttccgctgtcaagtccagttctacgggctctcggagaatgacgagtggacccaggatagggccaaacctgtcacccagatcgtcagcgccgaggcctggggtagagcagactgtggcttcacctccgagtcttaccagcaaggggtcctgtctgccaccatcctctatgagatcttgctagggaaggccaccttgtatgccgtgctggtcagtgccctcgtgctgatggccatggtcaagagaaaggattccagaggc

SEQ ID NO: 24 - protein, 309 aa, Artificial Sequence
  Artificially synthesized sequence
MGSRLFFVLSSLLCSKHMEAAVTQSPRNKVAVTGGKVTLSCNQTNNHNNMYWYRQDTGHGLRLIHYSYGAGSTEKGDIPDGYKASRPSQENFSLILELATPSQTSVYFCASGDTGGYEQYFGPGTRLTVLEDLKNVFPPEVAVFEPSEAEISHTQKATLVCLATGFYPDHVELSWWVNGKEVHSGVCTDPQPLKEQPALNDSRYCLSSRLRVSATFWQNPRNHFRCQVQFYGLSENDEWTQDRAKPVTQIVSAEAWGRADCGFTSESYQQGVLSATILYEILLGKATLYAVLVSALVLMAMVKRKDSRG

SEQ ID NO: 25 - DNA, 804 bp, Artificial Sequence
  Artificially synthesized sequence
atgcacagcctcctggggttgttgttgtggctgcaactgacaagggtgaatagtcaactagcagaagagaattcgtgggccctgagcgtccacgagggtgaaagtgtcacggtgaattgtagttacaagacatccataactgccctacagtggtacagacagaagtcaggcaaaggccctgcccagctaatcttaatacgttcaaatgagagagagaagcgcaatggaagactcagagccacccttgacacctccagccagagcagctccttgtccatcactgctactcggtgtgaagacaccgctgtgtacttctgtgccgcatcttctggcagctggcaactcatctttggatctggaacccaactgacagttatgcctgatatccagaaccctgaccctgccgtgtaccagctgagagactctaaatccagtgacaagtctgtctgcctattcaccgattttgattctcaaacaaatgtgtcacaaagtaaggattctgatgtgtatatcacagacaaatgcgtgctagacatgaggtctatggacttcaagagcaacagtgctgtggcctggagcaacaaatctgactttgcatgtgcaaacgccttcaacaacagcattattccagaagacaccttcttccccagcccagaaagttcctgtgatgtcaagctggtcgagaaaagctttgaaacagatacgaacctaaactttcaaaacctgtcagtgattgggttccgaatcctcctcctgaaagtggccgggtttaatctgctcatgacgctgcggctgtggtccagc

SEQ ID NO: 26 - protein, 268 aa, Artificial Sequence
  Artificially synthesized sequence
MHSLLGLLLWLQLTRVNSQLAEENSWALSVHEGESVTVNCSYKTSITALQWYRQKSGKGPAQLILIRSNEREKRNGRLRATLDTSSQSSSLSITATRCEDTAVYFCAASSGSWQLIFGSGTQLTVMPDIQNPDPAVYQLRDSKSSDKSVCLFTDFDSQTNVSQSKDSDVYITDKCVLDMRSMDFKSNSAVAWSNKSDFACANAFNNSIIPEDTFFPSPESSCDVKLVEKSFETDTNLNFQNLSVIGFRILLLKVAGFNLLMTLRLWSS

SEQ ID NO: 27 - DNA, 939 bp, Artificial Sequence
  Artificially synthesized sequence
atggcccccaggctccttttctgtctggttctttgcttcttgagagcagaaccaacaaatgctggtgtcatccaaacacctaggcacaaggtgacagggaagggacaagaagcaactctgtggtgtgagccaatttcaggacatagtgctgttttctggtacagacagaccattgtgcagggcctggagttcctgacttactttcgaaatcaagctcctatagatgattcagggatgcccaaggaacgattctcagctcagatgcccaatcagtcgcactcaactctgaagatccagagcacgcaaccccaggactcagcggtgtatctttgtgcaagcagcttagaagggacagtggaagaaacgctgtattttggctcaggaaccagactgactgttctcgaggacctgaaaaacgtgttcccacccgaggtcgctgtgtttgagccatcagaagcagagatctcccacacccaaaaggccacactggtgtgcctggccacaggcttctaccccgaccacgtggagctgagctggtgggtgaatgggaaggaggtgcacagtggggtctgcacagacccgcagcccctcaaggagcagcccgccctcaatgactccagatactgcctgagcagccgcctgagggtctcggccaccttctggcagaacccccgcaaccacttccgctgtcaagtccagttctacgggctctcggagaatgacgagtggacccaggatagggccaaacctgtcacccagatcgtcagcgccgaggcctggggtagagcagactgtggcttcacctccgagtcttaccagcaaggggtcctgtctgccaccatcctctatgagatcttgctagggaaggccaccttgtatgccgtgctggtcagtgccctcgtgctgatggccatggtcaagagaaaggattccagaggc

SEQ ID NO: 28 - protein, 313 aa, Artificial Sequence
  Artificially synthesized sequence
MAPRLLFCLVLCFLRAEPTNAGVIQTPRHKVTGKGQEATLWCEPISGHSAVFWYRQTIVQGLEFLTYFRNQAPIDDSGMPKERFSAQMPNQSHSTLKIQSTQPQDSAVYLCASSLEGTVEETLYFGSGTRLTVLEDLKNVFPPEVAVFEPSEAEISHTQKATLVCLATGFYPDHVELSWWVNGKEVHSGVCTDPQPLKEQPALNDSRYCLSSRLRVSATFWQNPRNHFRCQVQFYGLSENDEWTQDRAKPVTQIVSAEAWGRADCGFTSESYQQGVLSATILYEILLGKATLYAVLVSALVLMAMVKRKDSRG

SEQ ID NO: 29 - DNA, 630 bp, Artificial Sequence
  Artificially synthesized sequence
catatgtgggttaatagccagcagaaagttcagcagagtccggaaagcctgatcgttccggaaggcggcatggccagcctgaattgcaccagcagcgatcgcaatgttgattacttctggtggtaccgccagcatagcggcaaaagcccgaaaatgctgatgagcatcttcagcaatggcgaaaaagaagaaggccgcttcaccgttcatctgaataaagccagtctgcataccagcctgcatatccgcgatagccagccgagcgatagcgccctgtacctgtgcgccgcccgcgatagcaattaccagctgatctggggcagcggcaccaaactgatcatcaaaccggatatccagaatccggatccggccgtttaccagctgcgcgatagcaaaagcagcgataaaagcgtttgcctgttcaccgatttcgatagccagaccaatgttagccagagcaaagatagcgatgtttacatcaccgataaatgcgttctggatatgcgcagcatggatttcaaaagcaatagcgccgttgcctggagcaataaaagcgatttcgcctgcgccaatgccttcaataatagcatcatcccggaagataccttcttcccgtctccggaaagcagc

SEQ ID NO: 30 - DNA, 738 bp, Artificial Sequence
  Artificially synthesized sequence
atgaaacatatggaagccgccgttacccagagcccgcgcaataaagttgccgttaccggcggcaaagttaccctgagctgcaatcagaccaataatcataataatatgtactggtaccgccaggataccggccatggcctgcgcctgatccattacagctacggcgccggcagcaccgaaaaaggcgatatcccggatggctacaaagccagccgcccgagccaggaaaatttcagcctgatcctggaactggccaccccgagccagaccagcgtttacttctgcgccagcggcgataccggcggctacgaacagtacttcggcccgggcacccgcctgaccgttctggaagatctgaaaaatgttttcccgccggaagttgccgttttcgaaccgagcgaagccgaaatcagccatacccagaaagccaccctggtttgcctggccaccggcttctacccggatcatgttgaactgagctggtgggttaatggcaaagaagttcatagcggcgtttgcaccgatccgcagccgctgaaagaacagccggccctgaatgatagccgctacgccctgagcagccgcctgcgcgttagcgccaccttctggcaggatccgcgcaatcatttccgctgccaggttcagttctacggcctgagcgaaaatgatgaatggacccaggatcgcgccaaaccggttacccagatcgttagcgccgaagcctggggccgcgccgat

SEQ ID NO: 31 - DNA, 624 bp, Artificial Sequence
  Artificially synthesized sequence
atgcgcgttaatagccagctggccgaagaaaatagctgggccctgagcgttcatgaaggcgaaagcgttaccgttaattgcagctacaaaaccagtatcaccgccctgcagtggtaccgccagaaaagcggcaaaggcccggcccagctgatcctgatccgcagcaatgaacgcgaaaaacgcaatggccgcctgcgcgccaccctggataccagcagccagagcagcagcctgtctatcaccgccacccgctgcgaagataccgccgtttacttctgcgccgccagcagcggcagctggcagctgatcttcggcagcggcacccagctgaccgttatgccggatatccagaatccggatccggccgtttaccagctgcgcgatagcaaaagcagcgataaaagcgtttgcctgttcaccgatttcgatagccagaccaatgttagccagagcaaagatagcgatgtttacatcaccgataaatgcgttctggatatgcgcagcatggatttcaaaagcaatagcgccgttgcctggagcaataaaagcgatttcgcctgcgccaatgccttcaataatagcatcatcccggaagataccttcttcccgagcccggaaagcagc

SEQ ID NO: 32 - DNA, 747 bp, Artificial Sequence
  Artificially synthesized sequence
atggaaccgaccaatgccggcgttatccagaccccgcgccataaagttaccggcaaaggccaggaagccaccctgtggtgcgaaccgatcagcggccacagtgccgttttctggtaccgccagaccatcgttcagggcctggaattcctgacctacttccgcaatcaggccccgatcgatgatagcggcatgccgaaagaacgcttcagcgcccagatgccgaatcagagccatagcaccctgaaaatccagagcacccagccgcaggacagcgccgtttacctgtgcgccagcagcctggaaggcaccgttgaagaaaccctgtacttcggcagcggcacccgcctgaccgttctggaagatctgaaaaatgttttcccgccggaagttgccgttttcgaaccgagcgaagccgaaatcagccatacccagaaagccaccctggtttgcctggccaccggcttctacccggatcatgttgaactgagctggtgggttaatggcaaagaagttcatagcggcgtttgcaccgatccgcagccgctgaaagaacagccggccctgaatgatagccgctacgccctgagcagccgcctgcgcgttagcgccaccttctggcaggatccgcgcaatcatttccgctgccaggttcagttctacggcctgagcgaaaatgatgaatggacccaggatcgcgccaaaccggttacccagatcgttagcgccgaagcctggggccgcgccgat

SEQ ID NO: 33 - protein, 15 aa, Artificial Sequence
  Artificially synthesized sequence
GLNDIFEAQKIEWHE

SEQ ID NO: 34 - protein, 9 aa, Artificial Sequence
  Artificially synthesized sequence
VVGAGGVGK

SEQ ID NO: 35 - protein, 9 aa, Artificial Sequence
  Artificially synthesized sequence
VVGAVGVGK

SEQ ID NO: 36 - protein, 9 aa, Artificial Sequence
  Artificially synthesized sequence
VVGADGVGK

SEQ ID NO: 37 - protein, 9 aa, Artificial Sequence
  Artificially synthesized sequence
VVGACGVGK

SEQ ID NO: 38 - protein, 10 aa, Artificial Sequence
  Artificially synthesized sequence
VVVGAGGVGK

SEQ ID NO: 39 - protein, 10 aa, Artificial Sequence
  Artificially synthesized sequence
VVVGAVGVGK

SEQ ID NO: 40 - protein, 10 aa, Artificial Sequence
  Artificially synthesized sequence
VVVGADGVGK

SEQ ID NO: 41 - protein, 10 aa, Artificial Sequence
  Artificially synthesized sequence
VVVGACGVGK

SEQ ID NO: 42 - protein, 18 aa, Artificial Sequence
  Artificially synthesized sequence
EGRGSLLTCGDVEENPGP

SEQ ID NO: 43 - protein, 274 aa, Artificial Sequence
  Artificially synthesized sequence
MSHSMRYFYTSVSRPGRGEPRFIAVGYVDDTQFVRFDSDAASQRMEPRAPWIEQEGPEYWDQETRNVKAQSQTDRVDLGTLRGYYNQSEDGSHTIQIMYGCDVGPDGRFLRGYRQDAYDGKDYIALNEDLRSWTAADMAAQITKRKWEAAHAAEQQRAYLEGRCVEWLRRYLENGKETLQRTDPPKTHMTHHPISDHEATLRCWALGFYPAEITLTWQRDGEDQTQDTELVETRPAGDGTFQKWAAVVVPSGEEQRYTCHVQHEGLPKPLTLRW

SEQ ID NO: 44 - DNA, 822 bp, Artificial Sequence
  Artificially synthesized sequence
atgagccatagcatgcgctatttttataccagcgtgagccgcccgggccgcggcgaaccgcgctttattgcggtgggctatgtggatgatacccagtttgtgcgctttgatagcgatgcggcgagccagcgcatggaaccgcgcgcgccgtggattgaacaggaaggcccggaatattgggatcaggaaacccgcaacgtgaaagcgcagagccagaccgatcgcgtggatctgggcaccctgcgcggctattataaccagagcgaagatggcagccataccattcagattatgtatggctgcgatgtgggcccggatggccgctttctgcgcggctatcgccaggatgcgtatgatggcaaagattatattgcgctgaacgaagatctgcgcagctggaccgcggcggatatggcggcgcagattaccaaacgcaaatgggaagcggcgcatgcggcggaacagcagcgcgcgtatctggaaggccgctgcgtggaatggctgcgccgctatctggaaaacggcaaagaaaccctgcagcgcaccgatccgccgaaaacccatatgacccatcatccgattagcgatcatgaagcgaccctgcgctgctgggcgctgggcttttatccggcggaaattaccctgacctggcagcgcgatggcgaagatcagacccaggataccgaactggtggaaacccgcccggcgggcgatggcacctttcagaaatgggcggcggtggtggtgccgagcggcgaagaacagcgctatacctgccatgtgcagcatgaaggcctgccgaaaccgctgaccctgcgctgg

SEQ ID NO: 45 - protein, 274 aa, Artificial Sequence
  Artificially synthesized sequence
MSHSMRYFFTSVSRPGRGEPRFIAVGYVDDTQFVRFDSDAASQRMEPRAPWIEQEGPEYWDQETRNVKAQSQTDRVDLGTLRGYYNQSEAGSHTIQIMYGCDVGSDGRFLRGYRQDAYDGKDYIALNEDLRSWTAADMAAQITKRKWEAAHEAEQLRAYLDGTCVEWLRRYLENGKETLQRTDPPKTHMTHHPISDHEATLRCWALGFYPAEITLTWQRDGEDQTQDTELVETRPAGDGTFQKWAAVVVPSGEEQRYTCHVQHEGLPKPLTLRW

SEQ ID NO: 46 - DNA, 822 bp, Artificial Sequence
  Artificially synthesized sequence
atgagccatagcatgcgctatttttttaccagcgtgagccgcccgggccgcggcgaaccgcgctttattgcggtgggctatgtggatgatacccagtttgtgcgctttgatagcgatgcggcgagccagcgcatggaaccgcgcgcgccgtggattgaacaggaaggcccggaatattgggatcaggaaacccgcaacgtgaaagcgcagagccagaccgatcgcgtggatctgggcaccctgcgcggctattataaccagagcgaagcgggcagccataccattcagattatgtatggctgcgatgtgggcagcgatggccgctttctgcgcggctatcgccaggatgcgtatgatggcaaagattatattgcgctgaacgaagatctgcgcagctggaccgcggcggatatggcggcgcagattaccaaacgcaaatgggaagcggcgcatgaagcggaacagctgcgcgcgtatctggatggcacctgcgtggaatggctgcgccgctatctggaaaacggcaaagaaaccctgcagcgcaccgatccgccgaaaacccatatgacccatcatccgattagcgatcatgaagcgaccctgcgctgctgggcgctgggcttttatccggcggaaattaccctgacctggcagcgcgatggcgaagatcagacccaggataccgaactggtggaaacccgcccggcgggcgatggcacctttcagaaatgggcggcggtggtggtgccgagcggcgaagaacagcgctatacctgccatgtgcagcatgaaggcctgccgaaaccgctgaccctgcgctgg

SEQ ID NO: 47 - protein, 100 aa, Artificial Sequence [sequence omitted]

SEQ ID NO: 48 - DNA, 300 bp, Artificial Sequence
  Artificially synthesized sequence
atgattcagcgcaccccgaaaattcaggtgtatagccgccatccggcggaaaacggcaaaagcaactttctgaactgctatgtgagcggctttcatccgagcgatattgaagtggatctgctgaaaaacggcgaacgcattgaaaaagtggaacatagcgatctgagctttagcaaagattggagcttttatctgctgtattataccgaatttaccccgaccgaaaaagatgaatatgcgtgccgcgtgaaccatgtgaccctgagccagccgaaaattgtgaaatgggatcgcgatatg